European Patent Specification EP 3 568 454 B1, published May 17, 2023. Title: PROCEDE ENZYMATIQUE D'ELIMINATION DU SULFITE. Applicant: Université de Lorraine. The sequence listing filed with the application follows.

SEQUENCE LISTING (15 sequences)

SEQ ID NO: 1 - DNA, 846 bp, Escherichia coli
atgtccacgacatggtttgtaggagccgactggctcgccgaacatattgatgacccggaaattcagattatcgatgcccgcatggcgtcgcctggacaggaggatcgtaacgttgctcaggagtatctgaatggacatattcccggcgcagtgttttttgatatcgaagcgctttctgatcacacttccccgcttccgcacatgctgccgcgcccggaaacgttcgccgtggcgatgcgtgaattaggcgttaaccaggataagcacctgattgtctatgacgaaggtaatcttttctcagccccacgagcatggtggatgctgcgcacctttggtgtagagaaagtgtcgattctggggggtggacttgcaggctggcagcgcgatgatctgctgttagaagaaggtgcagtagagctgccggaaggagagtttaacgccgcgtttaatcctgaagccgtggtgaaagtaaccgatgtattattggcaagccatgaaaatacggcgcaaattattgatgcccgcccggctgcacgttttaacgcagaagttgatgaacctcgcccaggtttacgtcgcggacatattcccggagcactgaatgttccgtggacggaactggtgcgcgaaggcgaactaaaaacgaccgatgaactggatgcgatattttttggtcgcggcgtcagctacgacaaaccaattatcgtcagctgcggctctggtgtaacggcagccgtggttttgttagcactcgcgacgctggatgtgccaaacgtgaaactgtacgacggcgcatggagtgaatggggcgcgcgggcagatttaccggttgagccagtgaaataa

SEQ ID NO: 2 - protein, 281 aa, Escherichia coli
MSTTWFVGADWLAEHIDDPEIQIIDARMASPGQEDRNVAQEYLNGHIPGAVFFDIEALSDHTSPLPHMLPRPETFAVAMRELGVNQDKHLIVYDEGNLFSAPRAWWMLRTFGVEKVSILGGGLAGWQRDDLLLEEGAVELPEGEFNAAFNPEAVVKVTDVLLASHENTAQIIDARPAARFNAEVDEPRPGLRRGHIPGALNVPWTELVREGELKTTDELDAIFFGRGVSYDKPIIVSCGSGVTAAVVLLALATLDVPNVKLYDGAWSEWGARADLPVEPVK

SEQ ID NO: 3 - DNA, 33 bp, Artificial Sequence
  amorce sens
gccgaacatattgatgcgccggaaattcagatt

SEQ ID NO: 4 - DNA, 33 bp, Artificial Sequence
  amorce anti-sens
aatctgaatttccggcgcatcaatatgttccgc

SEQ ID NO: 5 - protein, 281 aa, Artificial Sequence
  Séquence protéique de la 3-MST Escherichia coli D17A
MSTTWFVGADWLAEHIDAPEIQIIDARMASPGQEDRNVAQEYLNGHIPGAVFFDIEALSDHTSPLPHMLPRPETFAVAMRELGVNQDKHLIVYDEGNLFSAPRAWWMLRTFGVEKVSILGGGLAGWQRDDLLLEEGAVELPEGEFNAAFNPEAVVKVTDVLLASHENTAQIIDARPAARFNAEVDEPRPGLRRGHIPGALNVPWTELVREGELKTTDELDAIFFGRGVSYDKPIIVSCGSGVTAAVVLLALATLDVPNVKLYDGAWSEWGARADLPVEPVK

SEQ ID NO: 6 - protein, 297 aa, Homo sapiens
MASPQLCRALVSAQWVAEALRAPRAGQPLQLLDASWYLPKLGRDARREFEERHIPGAAFFDIDQCSDRTSPYDHMLPGAEHFAEYAGRLGVGAATHVVIYDASDQGLYSAPRVWWMFRAFGHHAVSLLDGGLRHWLRQNLPLSSGKSQPAPAEFRAQLDPAFIKTYEDIKENLESRRFQVVDSRATGRFRGTEPEPRDGIEPGHIPGTVNIPFTDFLSQEGLEKSPEEIRHLFQEKKVDLSKPLVATCGSGVTACHVALGAYLCGKPDVPIYDGSWVEWYMRARPEDVISEGRGKTH

SEQ ID NO: 7 - protein, 370 aa, Leishmania major
MSAPAAAPKHPGKVFLDPSEVKDHLAEYRIVDCRYSLKIKDHGSIQYAKEHVKSAIRADVDTNLSKLVPTSTARHPLPPCAEFIDWCMANGMAGELPVLCYDDECGAMGGCRLWWMLNSLGADAYVINGGFQACKAAGLEMESGEPSSLPRPATHWPFKTAFQHHYLVDEIPPNAIITDARSADRFASTVRPYAADKMPGHIEGARNLPYTSHLVTRGDGKVLRSEEEIRHNIMTVVQGAGDAADLSSFVFSCGSGVTACINIALVHHLGLGHPYLYCGSWSEYSGLFRPPIMRSIIDDYGMCMQMQTPSLGDNPKANLDTMTLKVDGAPCERPDAEVQSAATHLHAGEAATVYFKSGRVVTIEVPAVPN

SEQ ID NO: 8 - DNA, 846 bp, Artificial Sequence
  Séquence du gène 3mst Escherichia coli D17A
atgtccacgacatggtttgtaggagccgactggctcgccgaacatattgatgcgccggaaattcagattatcgatgcccgcatggcgtcgcctggacaggaggatcgtaacgttgctcaggagtatctgaatggacatattcccggcgcagtgttttttgatatcgaagcgctttctgatcacacttccccgcttccgcacatgctgccgcgcccggaaacgttcgccgtggcgatgcgtgaattaggcgttaaccaggataagcacctgattgtctatgacgaaggtaatcttttctcagccccacgagcatggtggatgctgcgcacctttggtgtagagaaagtgtcgattctggggggtggacttgcaggctggcagcgcgatgatctgctgttagaagaaggtgcagtagagctgccggaaggagagtttaacgccgcgtttaatcctgaagccgtggtgaaagtaaccgatgtattattggcaagccatgaaaatacggcgcaaattattgatgcccgcccggctgcacgttttaacgcagaagttgatgaacctcgcccaggtttacgtcgcggacatattcccggagcactgaatgttccgtggacggaactggtgcgcgaaggcgaactaaaaacgaccgatgaactggatgcgatattttttggtcgcggcgtcagctacgacaaaccaattatcgtcagctgcggctctggtgtaacggcagccgtggttttgttagcactcgcgacgctggatgtgccaaacgtgaaactgtacgacggcgcatggagtgaatggggcgcgcgggcagatttaccggttgagccagtgaaataa

SEQ ID NO: 9 - DNA, 846 bp, Artificial Sequence
  Séquence du gène 3mst Escherichia coli pour la production dans l'hôte E. coli
atgagcaccacctggtttgttggtgcagattggctggcagaacatattgatgatccggaaattcagattatcgatgcacgtatggcaagtccgggtcaagaagatcgtaacgttgcacaagaatatctgaatggtcatattccgggtgccgtgttttttgatattgaagcactgagcgatcataccagtccgctgccgcatatgctgcctcgtccggaaacctttgcagttgcaatgcgtgaactgggtgttaatcaggataaacatctgatcgtgtatgatgaaggtaacctgtttagcgcaccgcgtgcatggtggatgctgcgtacctttggtgttgaaaaagttagcattttaggtggtggtctggcaggttggcagcgtgatgatctgctgctggaagaaggtgcagttgaactgccggaaggtgaatttaatgcagcatttaatccggaagccgttgttaaagttaccgatgttctgctggcaagccatgaaaataccgcacagatcattgatgcccgtccggcagcacgttttaatgccgaagttgatgaaccgcgtccgggtctgcgtcgtggccatattcctggcgcactgaatgttccgtggaccgaactggttcgtgaaggtgaactgaaaaccaccgatgaactggatgcaatcttttttggtcgtggtgtgagctatgataaaccgattattgttagctgtggtagcggtgttaccgcagcagttgtgctgctggcactggcaaccctggatgttccgaatgttaaactgtatgatggtgcatggtcagaatggggtgcacgtgccgatctgccggttgaaccggttaaataa

SEQ ID NO: 10 - DNA, 846 bp, Artificial Sequence
  Séquence du gène 3mst Escherichia coli D17A pour la production dans l'hôte E. coli
atgagcaccacctggtttgttggtgcagattggctggcagaacatattgatgcgccggaaattcagattatcgatgcacgtatggcaagtccgggtcaagaagatcgtaacgttgcacaagaatatctgaatggtcatattccgggtgccgtgttttttgatattgaagcactgagcgatcataccagtccgctgccgcatatgctgcctcgtccggaaacctttgcagttgcaatgcgtgaactgggtgttaatcaggataaacatctgatcgtgtatgatgaaggtaacctgtttagcgcaccgcgtgcatggtggatgctgcgtacctttggtgttgaaaaagttagcattttaggtggtggtctggcaggttggcagcgtgatgatctgctgctggaagaaggtgcagttgaactgccggaaggtgaatttaatgcagcatttaatccggaagccgttgttaaagttaccgatgttctgctggcaagccatgaaaataccgcacagatcattgatgcccgtccggcagcacgttttaatgccgaagttgatgaaccgcgtccgggtctgcgtcgtggccatattcctggcgcactgaatgttccgtggaccgaactggttcgtgaaggtgaactgaaaaccaccgatgaactggatgcaatcttttttggtcgtggtgtgagctatgataaaccgattattgttagctgtggtagcggtgttaccgcagcagttgtgctgctggcactggcaaccctggatgttccgaatgttaaactgtatgatggtgcatggtcagaatggggtgcacgtgccgatctgccggttgaaccggttaaataa

SEQ ID NO: 11 - DNA, 894 bp, Homo sapiens
atggcttcgccgcagctctgccgcgcgctggtgtcggcgcaatgggtggcggaggcgctgcgggccccgcgcgctgggcagcctctgcagctgctggacgcctcctggtacctgccgaagctggggcgcgacgcgcgacgcgagttcgaggagcgccacatcccgggcgccgctttcttcgacatcgaccagtgcagcgaccgcacctcgccctacgaccacatgctgcccggggccgagcatttcgcggagtacgcaggccgcctgggcgtgggcgcggccacccacgtcgtgatctacgacgccagcgaccagggcctctactccgccccgcgcgtctggtggatgttccgcgccttcggccaccacgccgtgtcactgcttgatggcggcctccgccactggctgcgccagaacctcccgctcagctccggcaagagccaacctgctcccgccgagttccgcgctcagctcgaccccgccttcatcaagacctacgaggacatcaaggagaacctggaatcccggcgcttccaggtggtggactcccgagccactggcaggttccgcggcaccgagcccgagccccgagacggcattgaacctggccacatcccaggtaccgtgaacatccccttcacagacttcctgagccaggaggggctggagaagagccctgaggagatccgccatctgttccaggagaagaaagtggacctgtctaagccactggtggccacgtgtggctctggcgtcacagcctgccacgtggcactaggggcctacctctgcggcaagccagacgtgcccatctacgatggctcctgggtggagtggtacatgcgcgcccggcccgaggatgtcatctcagagggccgggggaagacccactga

SEQ ID NO: 12 - DNA, 1113 bp, Leishmania major
atgtctgctcctgctgctgcgccgaaacacccgggcaaggtgttcctggacccgagcgaggtaaaggaccaccttgctgagtaccgcatcgtggactgccggtacagcttgaagataaaggaccacggcagcatccagtacgcgaaggagcacgtgaagagcgccatccgcgccgatgtggatacgaacctctctaagttggtgcccaccagcaccgcccggcatccgctaccgccctgtgctgagtttatcgactggtgcatggcgaacgggatggcgggagagctgccagtgctctgctacgatgacgagtgcggcgccatgggtggatgccgcctgtggtggatgctgaactctcttggcgccgacgcgtacgtgatcaacggcggctttcaggcctgcaaggctgcggggctggagatggagtccggcgagccctcgtcgctgccaagacccgcaacgcactggcccttcaagacggcctttcagcatcactaccttgtggatgaaatcccgcccaacgcaatcatcaccgacgcgcgctccgccgaccgcttcgcctcgacagtacgaccttacgccgcagacaagatgccaggccacatcgaaggtgcgcgtaacctcccctacacgtcgcacctcgtgacacgcggtgacggcaaggtgctgcgcagtgaggaagagatccgccacaacatcatgaccgtcgtgcaaggcgcgggtgacgcggctgatctatcgagcttcgtcttctcctgcggcagcggcgtcaccgcctgcatcaatatcgccctggtgcaccacctcggcctgggccatccgtacctctactgtggctcctggtctgagtacagcggcctcttccgcccccccataatgcgcagcatcatcgacgactacggcatgtgcatgcaaatgcagacccctagcctcggcgacaacccgaaggcaaacctcgacaccatgacgctgaaggtcgacggcgcgccctgcgagagacccgatgcggaggtgcagagcgccgcaacccacctccacgctggcgaggccgctaccgtgtacttcaagagcggccgcgtcgtcacgatcgaggtgccggcagtgcccaactaa

SEQ ID NO: 13 - protein, 5 aa, Artificial Sequence
  partie de séquence de la 3-mercaptopyruvate sulfurtransférase
  MISC_FEATURE (2)..(2): Xaa est A, V ou L
RXWWM

SEQ ID NO: 14 - protein, 8 aa, Artificial Sequence
  partie de séquence de la 3-mercaptopyruvate sulfurtransférase
  MISC_FEATURE (8)..(8): Xaa est A ou C
CGSGVTAX

SEQ ID NO: 15 - protein, 5 aa, Artificial Sequence
  partie de séquence de 3-mercaptopyruvate sulfurtransférase
  MISC_FEATURE (4)..(4): Xaa est est P ou E
GHIXG